European Patent Specification EP 3 458 049 B1, published March 5, 2025. Title: METHODS OF TREATING SEPSIS WITH SYNAPTIC VESICLE 2A BINDING CHEMICAL ENTITIES. Applicant: INSTITUT PASTEUR. The sequence listing filed with the application follows.

SEQUENCE LISTING (58 sequences)

SEQ ID NO: 1 - DNA, 20 bp, artificial sequence
  synthetic oligonucleotide
ctggaagaagctgccaaaac

SEQ ID NO: 2 - DNA, 20 bp, artificial sequence
  synthetic oligonucleotide
ccaatgccaagggagactaa

SEQ ID NO: 3 - DNA, 20 bp, artificial sequence
  synthetic oligonucleotide
gagcgggatagtaacgctga

SEQ ID NO: 4 - DNA, 20 bp, artificial sequence
  synthetic oligonucleotide
ggctctcactgccttcactc

SEQ ID NO: 5 - DNA, 21 bp, artificial sequence
  synthetic oligonucleotide
tcattcaccagacagattgct

SEQ ID NO: 6 - DNA, 20 bp, artificial sequence
  synthetic oligonucleotide
aagcgtttgcggtactcatt

SEQ ID NO: 7 - DNA, 20 bp, artificial sequence
  synthetic oligonucleotide
tacacagcaccagtccaagc

SEQ ID NO: 8 - DNA, 20 bp, artificial sequence
  synthetic oligonucleotide
agaaataaaggcccgtgtcc

SEQ ID NO: 9 - DNA, 20 bp, artificial sequence
  synthetic oligonucleotide
cttcgggcctttggaataat

SEQ ID NO: 10 - DNA, 20 bp, artificial sequence
  synthetic oligonucleotide
tagaagagcccttgggttga

SEQ ID NO: 11 - DNA, 20 bp, artificial sequence
  synthetic oligonucleotide
gtgaagaacccacggtctgt

SEQ ID NO: 12 - DNA, 20 bp, artificial sequence
  synthetic oligonucleotide
gccagagatgcttccaactg

SEQ ID NO: 13 - DNA, 20 bp, artificial sequence
  synthetic oligonucleotide
gatcacaatcatgggcacag

SEQ ID NO: 14 - DNA, 20 bp, synthetic oligonucleotide
attgaagcgggggttaaagt

SEQ ID NO: 15 - DNA, 20 bp, artificial sequence
  synthetic oligonucleotide
tggatgctcttcagttcgtg

SEQ ID NO: 16 - DNA, 20 bp, artificial sequence
  synthetic oligonucleotide
gcaacactcatccacaatgc

SEQ ID NO: 17 - DNA, 20 bp, artificial sequence
  synthetic oligonucleotide
gccaggacagttacctttgg

SEQ ID NO: 18 - DNA, 21 bp, artificial sequence
  synthetic oligonucleotide
ttcctggtagagaggcaaaca

SEQ ID NO: 19 - DNA, 21 bp, artificial sequence
  synthetic oligonucleotide
cttttgacgtcactggagttg

SEQ ID NO: 20 - DNA, 19 bp, artificial sequence
  synthetic oligonucleotide
cagtgagcgctgaatcgaa

SEQ ID NO: 21 - DNA, 20 bp, artificial sequence
  synthetic oligonucleotide
aagttcccttcccatctgct

SEQ ID NO: 22 - DNA, 20 bp, artificial sequence
  synthetic oligonucleotide
ggacaggaagatggttccaa

SEQ ID NO: 23 - DNA, 20 bp, artificial sequence
  syntehtic oligonucleotide
tccagaaacccctgtgtagc

SEQ ID NO: 24 - DNA, 20 bp, artificial sequence
  synthetic oligonucleotide
cagcagtgtgcagttgatga

SEQ ID NO: 25 - DNA, 19 bp, artificial sequence
  synthetic oligonucleotide
caggggttaagcctgagtg

SEQ ID NO: 26 - DNA, 19 bp, artificial sequence
  synthetic oligonucleotide
agtctggccgatcaaggag

SEQ ID NO: 27 - DNA, 20 bp, artificial sequence
  synthetic oligonucleotide
ttgtgccaagtctggagatg

SEQ ID NO: 28 - DNA, 20 bp, artificial sequence
  syntehtic oligoucleotide
ttctcagagcggatgaaggt

SEQ ID NO: 29 - DNA, 19 bp, artificial sequence
  synthetic oligonucleotide
ggataagcagacccgaagc

SEQ ID NO: 30 - DNA, 21 bp, artificial sequence
  synthetic oligonucleotide
actctggagagacttggttgg

SEQ ID NO: 31 - DNA, 20 bp, artificial sequence
  synthetic oligonucleotide
cggaaagtggaatccttgca

SEQ ID NO: 32 - DNA, 22 bp, artificial sequence
  synthetic oligonucleotide
cacatcgatctggacatgctgt

SEQ ID NO: 33 - DNA, 25 bp, artificial sequence
  synthetic oligonucleotide
gaccctcacactcagatcatcttct

SEQ ID NO: 34 - DNA, 20 bp, artificial sequence
  synthetic oligonucleotide
cctccacttggtggtttgct

SEQ ID NO: 35 - DNA, 22 bp, artificial sequence
  synthetic oligonucleotide
ctggtgtgtgcagttcccatta

SEQ ID NO: 36 - DNA, 18 bp, artificial sequence
  synthetic oligonucleotide
ccgacagcacgaggcttt

SEQ ID NO: 37 - DNA, 20 bp, artificial sequence
  synthetic oligonucleotide
caaactgatgaagctcgtca

SEQ ID NO: 38 - DNA, 20 bp, artificial sequence
  synthetic oligonucleotide
tctccttgagcgctcacgaa

SEQ ID NO: 39 - DNA, 20 bp, artificial sequence
  synthetic oligonucleotide
aagccaagcacgaagctaac

SEQ ID NO: 40 - DNA, 20 bp, artificial sequence
  synthetic oligonucleotide
atttgccgctctagggactc

SEQ ID NO: 41 - DNA, 23 bp, artificial sequence
  synthetic oligonucleotide
catcggcattttgaacgaggtca

SEQ ID NO: 42 - DNA, 22 bp, artificial sequence
  synthetic oligonucleotide
cttatcgatgaatcaggcatcg

SEQ ID NO: 43 - DNA, 25 bp, artificial sequence
  synthetic oligonucleotide
ccagttttacctggtagaagtgatg

SEQ ID NO: 44 - DNA, 28 bp, artificial sequence
  synthetic oligonucleotide
tgtctaggtcctggagtccagcagactc

SEQ ID NO: 45 - DNA, 20 bp, artificial sequence
  synthetic oligonucleotide
cccaatgagtaggctggaga

SEQ ID NO: 46 - DNA, 20 bp, artificial sequence
  synthetic oligonucleotide
tctggacccattccttcttg

SEQ ID NO: 47 - DNA, 25 bp, artificial sequence
  synthetic oligonucleotide
tgatgacatcaagaaggtggtgaag

SEQ ID NO: 48 - DNA, 23 bp, artificial sequence
  synthetic oligonucleotide
tccttggaggccatgtgggccat

SEQ ID NO: 49 - DNA, 20 bp, artificial sequence
  synthetic oligonucleotide
ctaaggccaaccgtgaaaag

SEQ ID NO: 50 - DNA, 20 bp, artificial sequence
  synthetic oligonucleotide
accagaggcatacagggaca

SEQ ID NO: 51 - DNA, 20 bp, artificial sequence
  synthetic oligonucleotide
cggacaggattgacagattg

SEQ ID NO: 52 - DNA, 20 bp, artificial sequence
  synthetic oligonucleotide
caaatcgctccaccaactaa

SEQ ID NO: 53 - DNA, 18 bp, artificial sequence
  synthetic oligonucleotide
ggccttccgtgttcctac

SEQ ID NO: 54 - DNA, 21 bp, artificial sequence
  synthetic oligonucleotide
tgtcatcatatctggcaggtt

SEQ ID NO: 55 - DNA, 22 bp, artificial sequence
  synthetic oligonucleotide
cccttcaatggttggtacatgg

SEQ ID NO: 56 - DNA, 21 bp, artificial sequence
  synthetic oligonucleotide
acattgatctccgtgacagcc

SEQ ID NO: 57 - DNA, 21 bp, artificial sequence
  synthetic oligonucleotide
caaagccagagtccttcagag

SEQ ID NO: 58 - DNA, 20 bp, synthetic oligonucleotide
tggtccttagccactccttc